European Patent Application EP 4 163 386 A1, published April 12, 2023. Title: COMBINATION OF GENE MARKERS AND USE THEREOF. Applicant: CREATIVE BIOSCIENCES (GUANGZHOU) CO., LTD. Application EP20939371.9. The sequence listing filed with the application follows.

SEQUENCE LISTING (22 sequences)

SEQ ID NO: 1 - DNA, 22 bp, Artificial Sequence
  HOXB4 primer F
ttcgtcgttttcgttatcattc

SEQ ID NO: 2 - DNA, 18 bp, Artificial Sequence
  HOXB4 primer R
tactaaccgcctcgctac

SEQ ID NO: 3 - DNA, 24 bp, Artificial Sequence
  HOXB4 probe P
cgggtttttgcgtcgttattcgtc

SEQ ID NO: 4 - DNA, 20 bp, Artificial Sequence
  SRCIN1 primer F
tcgtgtgtcgtcgttcagac

SEQ ID NO: 5 - DNA, 21 bp, Artificial Sequence
  SRCIN1 primer R
gaaatacccgcgaaaatactg

SEQ ID NO: 6 - DNA, 24 bp, Artificial Sequence
  SRCIN1 probe P
agttttacgttggagaagcgtcgg

SEQ ID NO: 7 - DNA, 21 bp, Artificial Sequence
  PCDHGA12 forward primer
ttggtttttacggttttcgac

SEQ ID NO: 8 - DNA, 19 bp, Artificial Sequence
  PCDHGA12 reverse primer
aaattctccgaaacgctcg

SEQ ID NO: 9 - DNA, 24 bp, Artificial Sequence
  PCDHGA12 probe
attcggtgcgtataggtatcgcgc

SEQ ID NO: 10 - DNA, 18 bp, Artificial Sequence
  HOXD8 forward primer
ttagtttcggcgcgtagc

SEQ ID NO: 11 - DNA, 20 bp, Artificial Sequence
  HOXD8 reverse primer
cctaaaaccgacgcgatcta

SEQ ID NO: 12 - DNA, 25 bp, Artificial Sequence
  HOXD8 probe
aaaacttacgatcgtctaccctccg

SEQ ID NO: 13 - DNA, 25 bp, Artificial Sequence
  beta-actin forward primer
ggaggtttagtaagttttttggatt

SEQ ID NO: 14 - DNA, 23 bp, Artificial Sequence
  beta-actin reverse primer
caataaaacctactcctccctta

SEQ ID NO: 15 - DNA, 20 bp, Artificial Sequence
  beta-actin probe
ttgtgtgttgggtggtggtt

SEQ ID NO: 16 - DNA, 20 bp, Artificial Sequence
  HOXB4 forward primer
attcgttcgggtattacgtc

SEQ ID NO: 17 - DNA, 19 bp, Artificial Sequence
  HOXB4 reverse primer
ccaaaatcccgacaaaccg

SEQ ID NO: 18 - DNA, 24 bp, Artificial Sequence
  HOXB4 detection probe
cggttagaggcgagagagtagttt

SEQ ID NO: 19 - DNA, 19 bp, Artificial Sequence
  HOXB4 forward primer
cgggtttcgggcggcgcgc

SEQ ID NO: 20 - DNA, 21 bp, Artificial Sequence
  HOXB4 reverse primer
cgaacgataacgaaaacgacg

SEQ ID NO: 21 - DNA, 27 bp, Artificial Sequence
  HOXB4 detection probe
amcgtgtatcgtgtagcgttacgcggb

SEQ ID NO: 22 - DNA, 22 bp, Artificial Sequence
  SRCIN1 forward primer
tatcgtgtatcgtcgttcggac